European Patent Application EP 4 567 116 A1, published June 11, 2025. Title: OPTICAL SWITCH PROTEIN THAT FUNCTIONS THROUGH IRRADIATION WITH LONG WAVELENGTH LIGHT. Applicant: 国立大学法人　東京大学. Application EP 23 850 081.3, filed August 1, 2023. The sequence listing filed with the application follows.

SEQUENCE LISTING (11 sequences)

SEQ ID NO: 1 - protein, 730 aa, Rhodopseudomonas palustris
MVAGHASGSPAFGTADLSNCEREEIHLAGSIQPHGALLVVSEPDHRIIQASANAAEFLNLGSVLGVPLAEIDGDLLIKILPHLDPTAEGMPVAVRCRIGNPSTEYDGLMHRPPEGGLIIELERAGPPIDLSGTLAPALERIRTAGSLRALCDDTALLFQQCTGYDRVMVYRFDEQGHGEVFSERHVPGLESYFGNRYPSSDIPQMARRLYERQRVRVLVDVSYQPVPLEPRLSPLTGRDLDMSGCFLRSMSPIHLQYLKNMGVRATLVVSLVVGGKLWGLVACHHYLPRFIHFELRAICELLAEAIATRITALESFAQSQSELFVQRLEQRMIEAITREGDWRAAIFDTSQSILQPLHADGCALVYEDQIRTIGDVPSTQDVREIAGWLDRQPRAAVTSTASLGLDVPELAHLTRMASGVVAAPISDHRGEFLMWFRPERVHTVTWGGDPKKPFTMGDTPADLSPRRSFAKWHQVVEGTSDPWTAADLAAARTIGQTVADIVLQFRAVRTLIAREQYEQFSSQVHASMQPVLITDAEGRILLMNDSFRDMLPAGSPSAVHLDDLAGFFVESNDFLRNVAELIDHGRGWRGEVLLRGAGNRPLPLAVRADPVTRTEDQSLGFVLIFSDATDRRTADAARTRFLEGILASARPGVRLDSKSDLLHEKLLSALVENAQLAALEITYGVETGRIAELLEGVRQSMLRTAEVLGHLVQHAARTAGSDSSSNGSQN

SEQ ID NO: 2 - protein, 731 aa, Rhodopseudomonas palustris
MAGHASGSPAFGTADLSNCEREEIHLAGSIQPHGALLVVSEPDHRIIQASANAAEFLNLGSVLGVPLAEIDGDLLIKILPHLDPTAEGMPVAVRCRIGNPSTEYDGLMHRPPEGGLIIELERAGPPIDLSGTLAPALERIRTAGSLRALCDDTALLFQQCTGYDRVMVYRFDEQGHGEVFSERHVPGLESYFGNRYPSSDIPQMARRLYERQRVRVLVDVSYQPVPLEPRLSPLTGRDLDMSGCFLRSMSPIHLQYLKNMGVRATLVVSLVVGGKLWGLVACHHYLPRFIHFELRAICELLAEAIATRITALESFAQSQSELFVQRLEQRMIEAITREGDWRAAIFDTSQSILQPLHADGCALVYEDQIRTIGDVPSTQDVREIAGWLDRQPRAAVTSTASLGLDVPELAHLTRMASGVVAAPISDHRGEFLMWFRPERVHTVTWGGDPKKPFTMGDTPADLSPRRSFAKWHQVVEGTSDPWTAADLAAARTIGQTVADIVLQFRAVRTLIAREQYEQFSSQVHASMQPVLITDAEGRILLMNDSFRDMLPAGSPSAVHLDDLAGFFVESNDFLRNVAELIDHGRGWRGEVLLRGAGNRPLPLAVRADPVTRTEDQSLGFVLIFSDATDRRTADAARTRFQEGILASARPGVRLDSKSDLLHEKLLSALVENAQLAALEITYGVETGRIAELLEGVRQSMLRTAEVLGHLVQHAARTAGSDSSSNGSQNKK

SEQ ID NO: 3 - protein, 464 aa, Rhodopseudomonas palustris
MASKSVHADITLLLDMEGVIREATLSPTMAAESVDGWLGRRWSDIAGAEGGDKVRRMVEDARRSGISAFRQINQPFPSGVEIPIEFTTMLLGDRTGMIAVGKNMQAVTELHSRLIAAQQAMERDYWRLRELETRYRLVFDAAADAVMIVSAGDMRIVEANRAAVNAISRVERGNDDLAGRDFLAEVAAADRDAVRDMLAQVRQRGTALSVLVHLGRYDRAWMLRGSLMSSERRQVFLLHFTPVTTTPAIDDVDDDAVLRGLIDRIPDGFVALDSEGVVRHANQAFLDLVQIGSKPAAVGRSLGVWMGRPGADLSSLLTLLRRYKTVRLFQTTIRGELGTETEVEVSAVDGEDDQYIGVLMRNVARRLDAADDHDALRQALGPISKQLGRSSLRKLVKNAVSIVEQHYVKEALLRSKGNRTATAELLGLSRQSLYAKLNSYGFDDKGVVASAADGAEGASDDAED

SEQ ID NO: 4 - DNA, 2190 bp, Rhodopseudomonas palustris
  source 1..2190: mol_type = other DNA
atggtcgctggacacgcttctgggagccccgcctttgggactgccgatctgagtaactgcgagagggaggaaattcacctggccggatctatccagccacacggcgccctgctggtggtctcagaacccgaccatcgcatcattcaggcaagcgccaacgccgctgagttcctgaatctgggcagcgtgctgggggtccccctggccgaaatcgacggcgacctgctgatcaagattctgcctcacctggacccaaccgccgagggaatgcctgtggccgtcagatgcaggattgggaacccatccaccgaatacgatggactgatgcatcgaccacctgagggaggactgatcattgagctggaacgagcaggaccaccaatcgacctgagtgggacactggctcccgcactggaacgcattcgaactgccggatcactgcgggctctgtgcgacgatactgccctgctgttccagcagtgtaccggctacgacagagtgatggtctatcgcttcgatgagcagggccacggggaggtgttttctgaaagacatgtccctgggctggaaagttactttggaaacaggtatcctagctccgacatcccacagatggcccggagactgtacgagcggcagagagtgagggtcctggtggatgtcagctatcagcctgtgccactggaaccaaggctgtcccctctgaccggacgcgacctggatatgtctggctgcttcctgcgctcaatgagccccatccacctccagtacctgaagaatatgggggtgcgggccacactggtggtcagcctggtggtcggaggcaaactgtggggactggtggcctgccaccattatctgcctcgattcatccattttgagctgcgggctatttgtgagctgctggccgaagctatcgcaacccgcattacagcactggaatccttcgcccagtcccagtctgagctgtttgtgcagcgcctggagcagcgaatgatcgaagccattacccgagagggcgactggcgagcagcaatctttgatacaagtcagagcatcctccagcctctgcacgctgacggctgtgcactggtgtacgaggatcagatccgcaccattggggacgtgccaagcacacaggatgtccgggaaatcgcaggatggctggaccgacagccccgggccgccgtgaccagcaccgccagcctgggcctggatgtgccagagctggctcacctgaccagaatggcaagtggagtggtcgccgctcccatttcagaccacaggggcgagttcctgatgtggtttaggcctgagcgcgtgcatactgtcacctgggggggagatccaaagaaacccttcactatgggcgacacccccgctgatctgtcccctaggcgctcttttgcaaaatggcaccaggtggtcgagggcacttctgacccttggaccgcagccgatctggctgccgccagaacaatcgggcagactgtggccgacatcgtgctccagttccgggccgtgcggacactgatcgctagggagcagtatgaacagttttctagtcaggtgcatgccagcatgcagccagtcctgatcactgatgctgagggcagaatcctgctgatgaacgactccttcagggatatgctgccagctgggagcccatccgcagtgcacctggacgatctggcaggattctttgtggaaagcaacgactttctgagaaatgtcgctgagctgatcgaccatggaagaggctggaggggagaggtgctgctgagaggagcaggaaataggccactgcctctggcagtgcgggccgacccagtcacaagaactgaagatcagagcctgggcttcgtgctgatcttttccgacgcaaccgatcgacgaacagccgacgctgcacgaacccgattcctggagggcattctggcctctgctcgaccaggggtgagactggactctaagagtgatctgctgcacgaaaaactgctgagtgccctggtggagaatgctcagctggccgctctggaaatcacatatggagtggagactggcaggattgcagagctgctggaaggcgtgcgccagtccatgctgcgaacagctgaggtgctggggcatctggtccagcacgcagcacgcacagcagggagcgatagcagcagcaatgggagtcagaat

SEQ ID NO: 5 - DNA, 1392 bp, Rhodopseudomonas palustris
  source 1..1392: mol_type = other DNA
atggcatctaagtctgtgcacgctgacatcaccctgctgctggatatggaaggagtcattcgagaggctaccctgagcccaactatggccgctgaatctgtggacggatggctgggccggagatggagtgatatcgctggagcagaaggaggggacaaggtgaggcgaatggtcgaggatgcacgacggtccggaatctctgctttcaggcagattaatcagccctttcctagcggcgtggaaatccccattgagttcaccacaatgctgctgggagatcgcacaggcatgatcgcagtggggaaaaacatgcaggccgtcactgaactgcactccaggctgattgcagcccagcaggccatggagcgcgactactggaggctgcgcgagctggaaacccgatatcggctggtgttcgatgccgccgccgacgccgtgatgatcgtcagtgctggcgatatgaggattgtggaagctaaccgcgccgccgtgaatgcaatcagccgcgtcgagcgaggcaatgacgatctggcagggagggactttctggcagaggtggccgccgccgacagggacgctgtgcgcgatatgctggcacaggtcagacagaggggcacagccctgtccgtgctggtccacctggggcggtacgacagagcttggatgctgagaggatctctgatgagcagcgaaagaaggcaggtgttcctgctgcacttcaccccagtcactaccacacccgccatcgacgatgtggacgatgacgctgtcctgagaggcctgatcgacaggattcccgacggattcgtggccctggacagcgagggagtggtccggcatgcaaatcaggcctttctggatctggtgcagattggcagcaagcctgccgctgtggggaggtccctgggagtctggatggggcgcccaggagccgacctgtctagtctgctgactctgctgcgccgatacaaaaccgtgcggctgttccagactaccatcagaggcgaactggggacagagactgaagtggaggtctctgccgtggatggagaggatgaccagtatattggcgtgctgatgcggaacgtcgcccggagactggatgcagccgatgaccacgacgctctgagacaggcactggggcctatcagcaagcagctgggacgatcaagcctgcggaagctggtgaaaaacgcagtgtcaattgtcgaacagcattatgtgaaggaggctctgctgcgcagcaaaggcaatcgaaccgccacagctgagctgctggggctgagtcggcagtcactgtacgccaaactgaacagctatggctttgatgacaagggcgtcgtggctagtgctgccgatggggccgaaggcgcaagcgatgatgctgaagat

SEQ ID NO: 6 - protein, 146 aa, Rhodopseudomonas palustris
MASKSVHADITLLLDMEGVIREATLSPTMAAESVDGWLGRRWSDIAGAEGGDKVRRMVEDARRSGISAFRQINQPFPSGVEIPIEFTTMLLGDRTGMIAVGKNMQAVTELHSRLIAAQQAMERDYWRLRELETRYRLVFDAAADAV

SEQ ID NO: 7 - DNA, 20 bp, Homo sapiens
  source 1..20: mol_type = genomic DNA
gcagccgctcgctgcagcag

SEQ ID NO: 8 - DNA, 20 bp, Homo sapiens
  source 1..20: mol_type = genomic DNA
ggctagggatgaagaataaa

SEQ ID NO: 9 - DNA, 20 bp, Homo sapiens
  source 1..20: mol_type = genomic DNA
gcctgggctccggggcgttt

SEQ ID NO: 10 - DNA, 21 bp, Homo sapiens
  source 1..21: mol_type = genomic DNA
gtccttggccacttccccatc

SEQ ID NO: 11 - DNA, 20 bp, Homo sapiens
  source 1..20: mol_type = genomic DNA
agctgaggaggtgggggaag